European Patent Specification EP 3 851 450 B1, published November 27, 2024. Title: Chimeric antigen receptors and methods of use. Applicant: ETH Zürich. The sequence listing filed with the application follows.

SEQUENCE LISTING (45 sequences)

SEQ ID NO: 1 - DNA, 30 bp, Homo sapiens
acgccttctgtatgaaacagtttttcctcc

SEQ ID NO: 2 - protein, 8 aa, Artificial Sequence
  Linker
GGSGGSAQ

SEQ ID NO: 3 - protein, 11 aa, Artificial Sequence
  Linker
AQSGGSGGSAQ

SEQ ID NO: 4 - protein, 29 aa, Artificial Sequence
  Synthetic construct comprising gp61 peptide
  PEPTIDE (3)..(18): GP61 peptide
SGLNGPDIYKGVYQFKSVGSGGSGGSGDS

SEQ ID NO: 5 - protein, 29 aa, Artificial Sequence
  synthetic construct comprising ova peptide
  PEPTIDE (2)..(18): OVA peptide
SISQAVHAAHAEINEAGRGSGGSGGSGDS

SEQ ID NO: 6 - DNA, 42 bp, Artificial Sequence
  Oligonucleotide encoding random peptides used for MCR2 library
  misc_feature (4)..(9): n is a, c, g, or t
  misc_feature (13)..(18): n is a, c, g, or t
  misc_feature (22)..(24): n is a, c, g, or t
  misc_feature (28)..(33): n is a, c, g, or t
  misc_feature (37)..(39): n is a, c, g, or t
ggtnnnnnntwcnnnnnnbccnnnsccnnnnnnkccnnngga

SEQ ID NO: 7 - protein, 267 aa, Homo sapiens
  MISC_FEATURE (1)..(208): MHC2 alpha
  MISC_FEATURE (209)..(216): linker sequence
  MISC_FEATURE (217)..(267): TCR alpha
MPRSRALILGVLALTTMLSLCGGEDDIEADHVGTYGISVYQSPGDIGQYTFEFDGDELFYVDLDKKETVWMLPEFGQLASFDPQGGLQNIAVVKHNLGVLTKRSNSTPATNEAPQATVFPKSPVLLGQPNTLICFVDNIFPPVINITWLRNSKSVADGVYETSFFVNRDYSFHKLSYLTFIPSDDDIYDCKVEHWGLEEPVLKHWEPEGGSGGSAQSDVPCDATLTEKSFETDMNLNFQNLSVMGLRILLLKVAGFNLLMTLRLWSS

SEQ ID NO: 8 - protein, 287 aa, Homo sapiens
  SIGNAL (1)..(26): leader peptide
  MISC_FEATURE (27)..(28): insertion site of oligopeptides
  MISC_FEATURE (29)..(36): linker sequence
  MISC_FEATURE (37)..(228): MHC2 beta
  MISC_FEATURE (229)..(236): linker sequence
  MISC_FEATURE (237)..(287): TCR beta
MALQIPSLLLSAAVVVLMVLSSPRTEGGSGGSGGSGDSERHFVYQFMGECYFTNGTQRIRYVTRYIYNREEYVRYDSDVGEHRAVTELGRPDAEYWNSQPEILERTRAELDTVCRHNYEGPETHTSLRRLEQPNVVISLSRTEALNHHNTLVCSVTDFYPAKIKVRWFRNGQEETVGVSSTQLIRNGDWTFQVLVMLEMTPRRGEVYTCHVEHPSLKSPITVEWRAQSGGSGGSAQGRADCGITSASYQQGVLSATILYEILLGKATLYAVLVSTLVVMAMVKRKNS

SEQ ID NO: 9 - protein, 16 aa, Lymphocytic choriomeningitis virus
LNGPDIYKGVYQFKSV

SEQ ID NO: 10 - protein, 17 aa, Gallus gallus
ISQAVHAAHAEINEAGR

SEQ ID NO: 11 - DNA, 49 bp, Lymphocytic choriomeningitis virus
ctgaatggtcctgacatttataagggtgtgtatcagtttaagtctgtgg

SEQ ID NO: 12 - DNA, 41 bp, Artificial Sequence
  altered gp61 sequence
ctgaatggtcctgccccgtgtgtatcagtttaagtctgtgg

SEQ ID NO: 13 - DNA, 49 bp, Artificial Sequence
  altered gp61 sequence
ctgaatggtcctgacattttcgcccgtgtgtatcagtttaagtctgtgg

SEQ ID NO: 14 - protein, 16 aa, Artificial Sequence
  amino acid sequence of SEQ ID NO 013
LNGPDIFARVYQFKSV

SEQ ID NO: 15 - DNA, 44 bp, Artificial Sequence
  altered gp61 sequence
ctgaatggtcctgacatccggtgtgtatcagtttaagtctgtgg

SEQ ID NO: 16 - DNA, 48 bp, Artificial Sequence
  altered gp61 sequence
vtgaatggtcctgacatttataaggggtgtatcagtttaagtctgtgg

SEQ ID NO: 17 - DNA, 43 bp, Artificial Sequence
  altered gp61 sequence
ctgaatggtcctgacatttgtgtgtatcagtttaagtctgtgg

SEQ ID NO: 18 - protein, 14 aa, Artificial Sequence
  amino acid sequence of SEQ ID NO 17
LNGPDICVYQFKSV

SEQ ID NO: 19 - DNA, 52 bp, Artificial Sequence
  altered gp61 sequence
ctgaatggtcctgacatttataagcgaattgtgtatcagtttaagtctgtgg

SEQ ID NO: 20 - protein, 17 aa, Artificial Sequence
  amino acid sequence of SEQ ID NO 019
LNGPDIYKRIVYQFKSV

SEQ ID NO: 21 - DNA, 41 bp, Artificial Sequence; identical to SEQ ID NO: 12
  altered gp61 sequence

SEQ ID NO: 22 - DNA, 48 bp, Artificial Sequence
  altered gp61 sequence
ctgaatggtcctgacatttccgcggtgtgtatcagtttaagtctgtgg

SEQ ID NO: 23 - DNA, 50 bp, Artificial Sequence
  altered gp61 sequence
ctgaatggtcctgacatttataatcggtgtgtatcagtttaagtctgtgg

SEQ ID NO: 24 - DNA, 45 bp, Artificial Sequence
  altered gp61 sequence
ctgaatggtcctgacattcccgtgtgtatcagtttaagtctgtgg

SEQ ID NO: 25 - DNA, 49 bp, Artificial Sequence
  altered gp61 sequence
ctgaatggtcctgacatttactccggtgtgtatcagtttaagtctgtgg

SEQ ID NO: 26 - protein, 16 aa, Artificial Sequence
  amino acid sequence of SEQ ID NO 025
LNGPDIYSGVYQFKSV

SEQ ID NO: 27 - DNA, 49 bp, Artificial Sequence
  altered gp61 sequence
ctgaatggtcctgacatttataatggtgtgtatcagtttaagtctgtgg

SEQ ID NO: 28 - protein, 16 aa, Artificial Sequence
  amino acid sequence of SEQ ID NO 027
LNGPDIYNGVYQFKSV

SEQ ID NO: 29 - DNA, 21 bp, Artificial Sequence
  example for coding sequence of random peptide
aacgatcgagctgcatgctac

SEQ ID NO: 30 - DNA, 21 bp, Artificial Sequence
  example for coding sequence of random peptide
acgatcgagctgcatgctaca

SEQ ID NO: 31 - DNA, 21 bp, Artificial Sequence
  example for coding sequence of random peptide
cgatcgagctgcatgctacag

SEQ ID NO: 32 - DNA, 21 bp, Artificial Sequence
  example for coding sequence of random peptide
gatcgagctgcatgctacagc

SEQ ID NO: 33 - DNA, 45 bp, Artificial Sequence
  nucleic acid sequence of dominant NP311 epitope
gaggggtggccatacatagcttgtagaacatcagttgtagggaga

SEQ ID NO: 34 - protein, 15 aa, Artificial Sequence
  amino acid sequence of SEQ ID NO 033
EGWPYIACRTSVVGR

SEQ ID NO: 35 - DNA, 30 bp, Artificial Sequence
  nucleic acid sequence of new NP547 epitope
gacctgatcttcagaggtccaaatgtggtg

SEQ ID NO: 36 - protein, 10 aa, Artificial Sequence
  amino acid sequence of SEQ ID NO 035
DLIFRGPNVV

SEQ ID NO: 37 - protein, 14 aa, Artificial Sequence
  random peptide example
  MISC_FEATURE (2)..(2): any amino acid
  MISC_FEATURE (3)..(3): any amino acid
  MISC_FEATURE (4)..(4): tyrosine or phenylalanine
  MISC_FEATURE (5)..(5): any amino acid
  MISC_FEATURE (6)..(6): any amino acid
  MISC_FEATURE (7)..(7): proline, alanine or serine
  MISC_FEATURE (8)..(8): any amino acid
  MISC_FEATURE (9)..(9): alanine or proline
  MISC_FEATURE (10)..(10): any amino acid
  MISC_FEATURE (11)..(11): any amino acid
  MISC_FEATURE (12)..(12): alanine or serine
  MISC_FEATURE (13)..(13): any amino acid
GXXXXXXXXXXXXG

SEQ ID NO: 38 - protein, 14 aa, Artificial Sequence
  random peptide
GGGYSASCPVIAPG

SEQ ID NO: 39 - protein, 13 aa, Artificial Sequence
  random peptide
GRRYKATASIAFG

SEQ ID NO: 40 - protein, 14 aa, Artificial Sequence
  random peptide
GNIFFISTASIANG

SEQ ID NO: 41 - protein, 14 aa, Artificial Sequence
  random peptide
GTMFLNASPGNSEG

SEQ ID NO: 42 - protein, 13 aa, Artificial Sequence
  random peptide
GTDYLSAARSSDG

SEQ ID NO: 43 - protein, 14 aa, Artificial Sequence
  random peptide
GGRYHRPLPCASPG

SEQ ID NO: 44 - protein, 14 aa, Artificial Sequence
  random peptide
GRGYISAYPHFSIG

SEQ ID NO: 45 - protein, 14 aa, Artificial Sequence
  random peptide
GGIFNRALPAPSKG